European Patent Application EP 4 269 442 A1, published November 1, 2023. Title: MESOTHELIN BINDING MOLECULE AND APPLICATION THEREOF. Applicant: ZHEJIANG NANOMAB TECH CENTER CO LTD. The sequence listing filed with the application follows.

SEQUENCE LISTING (125 sequences)

SEQ ID NO: 1 - protein, 11 aa, Artificial Sequence
  MSLN CDR1
  MISC_FEATURE (1)..(1): Xaa is Gly, Glu, Thr or Ala
  MISC_FEATURE (2)..(2): Xaa is Ser, Asn, Pro, Ala, His, Asp, Lys, Ile or Phe
  MISC_FEATURE (3)..(3): Xaa is Ile, Ser, Val, Thr, Asp, Leu, Ala, Met or His
  MISC_FEATURE (4)..(4): Xaa is Phe, Ser, Ile, Ala, Leu or Gly
  MISC_FEATURE (5)..(5): Xaa is Asn, Ser, Gly, Ala, Asp, Thr, Glu, Arg or His
  MISC_FEATURE (6)..(6): Xaa is Ile, Leu, Phe, Tyr, Glu or Asn
  MISC_FEATURE (7)..(7): Xaa is Asn, Ala, Gly, Asp, Lys, Tyr, Leu or Ser
  MISC_FEATURE (8)..(8): Xaa is Ala, Tyr, Val, Asp or Asn
  MISC_FEATURE (9)..(9): Xaa is Glu or null
  MISC_FEATURE (10)..(10): Xaa is Phe or null
  MISC_FEATURE (11)..(11): Xaa is Ala or null
XXXXXXXXXXX

SEQ ID NO: 2 - protein, 12 aa, Artificial Sequence
  MSLN CDR2
  MISC_FEATURE (1)..(1): Xaa is Ile, Met, Ala, Thr or Leu
  MISC_FEATURE (2)..(2): Xaa is Ser, Gly, Asn, Asp, Thr or Val
  MISC_FEATURE (3)..(3): Xaa is Ser, Asn, Ala, Arg, Gly or Thr
  MISC_FEATURE (4)..(4): Xaa is Ser, Thr, Gly, Asp or Asn
  MISC_FEATURE (5)..(5): Xaa is Asn, Gly, Thr or Ile
  MISC_FEATURE (6)..(6): Xaa is Ser, Arg, Asn, Asp, Lys, Thr or Gly
  MISC_FEATURE (7)..(7): Xaa is Asp, Thr, Ser, Ile or Lys
  MISC_FEATURE (8)..(8): Xaa is Asn, Thr, Gly, Asp or null
  MISC_FEATURE (9)..(9): Xaa is Thr, Lys, Gly or null
  MISC_FEATURE (10)..(10): Xaa is Gly, Arg or null
  MISC_FEATURE (11)..(11): Xaa is Val, Thr or null
  MISC_FEATURE (12)..(12): Xaa is Thr or null
XXXXXXXXXXXX

SEQ ID NO: 3 - protein, 23 aa, Artificial Sequence
  MSLN CDR3
  MISC_FEATURE (1)..(1): Xaa is Asn, His, Ala or Gln
  MISC_FEATURE (2)..(2): Xaa is Leu, Ala, Gly or Val
  MISC_FEATURE (3)..(3): Xaa is Ser, Arg, Glu, Gly, Asp or Thr
  MISC_FEATURE (4)..(4): Xaa is Asn, Ala, Arg, Gly, Asp, Lys, Val, Thr, Ile, Glu or Gln
  MISC_FEATURE (5)..(5): Xaa is Tyr, Phe, Lys, Ser, Cys, Ile, Asp, Gly, His or Arg
  MISC_FEATURE (6)..(6): Xaa is Asp, Ala, Val, Gly, Arg, Asn, Pro, Thr, Cys, Gln or Ser
  MISC_FEATURE (7)..(7): Xaa is Arg, Tyr, Thr, Ala, Asp, Lys, Leu, Glu, Ser or Gly
  MISC_FEATURE (8)..(8): Xaa is Lys, Ser, Phe, Thr, Asp, Gln, Glu, Gly, Pro, Arg, Tyr or Asn
  MISC_FEATURE (9)..(9): Xaa is Asp, Gly, Ile, His, Ser, Tyr, Gln, Lys, Thr, Arg or Val
  MISC_FEATURE (10)..(10): Xaa is Arg, Tyr, His, Asn, Thr, Asp, Pro, Val, Lys, Cys, Leu or Ser
  MISC_FEATURE (11)..(11): Xaa is Tyr, Asp, Glu, Pro, Phe, Ser, Leu, Ile or null
  MISC_FEATURE (12)..(12): Xaa is Pro, Val, Gln, Ala, Tyr, Phe, Asn, Asp, Arg or null
  MISC_FEATURE (13)..(13): Xaa is Asp, Ala, Tyr, Val, Gln, Pro or null
  MISC_FEATURE (14)..(14): Xaa is Tyr, Leu, Pro, Ala, Glu or null
  MISC_FEATURE (15)..(15): Xaa is Cys, Ser, Met, Pro, Thr or null
  MISC_FEATURE (16)..(16): Xaa is Val, Asp, Ser, Tyr or null
  MISC_FEATURE (17)..(17): Xaa is Leu, Phe, Val, Asp or null
  MISC_FEATURE (18)..(18): Xaa is Arg, Gly, Met, Ser or null
  MISC_FEATURE (19)..(19): Xaa is Asp, Asn, Ser or null
  MISC_FEATURE (20)..(20): Xaa is Tyr, Leu or null
  MISC_FEATURE (21)..(21): Xaa is Tyr or null
  MISC_FEATURE (22)..(22): Xaa is Ala or null
  MISC_FEATURE (23)..(23): Xaa is Asp or null
XXXXXXXXXXXXXXXXXXXXXXX

SEQ ID NO: 4 - protein, 8 aa, Artificial Sequence
  CDR1
GSIFNINA

SEQ ID NO: 5 - protein, 8 aa, Artificial Sequence
  CDR1
GNIFSINA

SEQ ID NO: 6 - protein, 8 aa, Artificial Sequence
  CDR1
ESISSIAY

SEQ ID NO: 7 - protein, 8 aa, Artificial Sequence
  CDR1
GSSFGLNV

SEQ ID NO: 8 - protein, 8 aa, Artificial Sequence
  CDR1
GSVSSINA

SEQ ID NO: 9 - protein, 8 aa, Artificial Sequence
  CDR1
GSTFAINA

SEQ ID NO: 10 - protein, 8 aa, Artificial Sequence
  CDR1
GSVIDIGA

SEQ ID NO: 11 - protein, 8 aa, Artificial Sequence
  CDR1
TPIISIAY

SEQ ID NO: 12 - protein, 8 aa, Artificial Sequence
  CDR1
GSIASIDA

SEQ ID NO: 13 - protein, 8 aa, Artificial Sequence
  CDR1
GAVSSINA

SEQ ID NO: 14 - protein, 8 aa, Artificial Sequence
  CDR1
EHTFTIDA

SEQ ID NO: 15 - protein, 8 aa, Artificial Sequence
  CDR1
GSDLSFDA

SEQ ID NO: 16 - protein, 8 aa, Artificial Sequence
  CDR1
GDSFGLNV

SEQ ID NO: 17 - protein, 8 aa, Artificial Sequence
  CDR1
ANLFTIDA

SEQ ID NO: 18 - protein, 8 aa, Artificial Sequence
  CDR1
GDAFSFDA

SEQ ID NO: 19 - protein, 8 aa, Artificial Sequence
  CDR1
GSLSSINA

SEQ ID NO: 20 - protein, 8 aa, Artificial Sequence
  CDR1
EKTFSIKY

SEQ ID NO: 21 - protein, 8 aa, Artificial Sequence
  CDR1
GISFEYYA

SEQ ID NO: 22 - protein, 8 aa, Artificial Sequence
  CDR1
GAVSTINA

SEQ ID NO: 23 - protein, 8 aa, Artificial Sequence
  CDR1
ASMGSISN

SEQ ID NO: 24 - protein, 8 aa, Artificial Sequence
  CDR1
GSHFGLNV

SEQ ID NO: 25 - protein, 8 aa, Artificial Sequence
  CDR1
GITLDNYA

SEQ ID NO: 26 - protein, 8 aa, Artificial Sequence
  CDR1
GFTFHYYA

SEQ ID NO: 27 - protein, 8 aa, Artificial Sequence
  CDR1
GSAFSFDA

SEQ ID NO: 28 - protein, 9 aa, Artificial Sequence
  CDR2
ISSSNSDNT

SEQ ID NO: 29 - protein, 9 aa, Artificial Sequence
  CDR2
ISSTNSDNT

SEQ ID NO: 30 - protein, 7 aa, Artificial Sequence
  CDR2
ISSTGST

SEQ ID NO: 31 - protein, 8 aa, Artificial Sequence
  CDR2
IGNGGRTT

SEQ ID NO: 32 - protein, 7 aa, Artificial Sequence
  CDR2
MGSGGNT

SEQ ID NO: 33 - protein, 8 aa, Artificial Sequence
  CDR2
ISSGGDST

SEQ ID NO: 34 - protein, 7 aa, Artificial Sequence
  CDR2
INAGGNT

SEQ ID NO: 35 - protein, 7 aa, Artificial Sequence
  CDR2
INSGGKT

SEQ ID NO: 36 - protein, 9 aa, Artificial Sequence
  CDR2
ISSSNSDNK

SEQ ID NO: 37 - protein, 7 aa, Artificial Sequence
  CDR2
AGRTGTT

SEQ ID NO: 38 - protein, 7 aa, Artificial Sequence
  CDR2
TSRDGRI

SEQ ID NO: 39 - protein, 7 aa, Artificial Sequence
  CDR2
ISSGGNK

SEQ ID NO: 40 - protein, 7 aa, Artificial Sequence
  CDR2
TSRDGRT

SEQ ID NO: 41 - protein, 7 aa, Artificial Sequence
  CDR2
MGSDGKT

SEQ ID NO: 42 - protein, 7 aa, Artificial Sequence
  CDR2
IDTDGKT

SEQ ID NO: 43 - protein, 12 aa, Artificial Sequence
  CDR2
TTSGTTSGGGVT

SEQ ID NO: 44 - protein, 11 aa, Artificial Sequence
  CDR2
LVATIGSDGRT

SEQ ID NO: 45 - protein, 8 aa, Artificial Sequence
  CDR2
IGNSGRTT

SEQ ID NO: 46 - protein, 7 aa, Artificial Sequence
  CDR2
ISSNGNT

SEQ ID NO: 47 - protein, 8 aa, Artificial Sequence
  CDR2
ISSSGDST

SEQ ID NO: 48 - protein, 11 aa, Artificial Sequence
  CDR3
AAENYDRKDRY

SEQ ID NO: 49 - protein, 11 aa, Artificial Sequence
  CDR3
AAENFDRKDRY

SEQ ID NO: 50 - protein, 13 aa, Artificial Sequence
  CDR3
AASNKAYNDYDPD

SEQ ID NO: 51 - protein, 10 aa, Artificial Sequence
  CDR3
HLRASVTKGY

SEQ ID NO: 52 - protein, 14 aa, Artificial Sequence
  CDR3
AADRFGASIHEVDY

SEQ ID NO: 53 - protein, 20 aa, Artificial Sequence
  CDR3
NARGCRDFHNPQALCVLRDY

SEQ ID NO: 54 - protein, 14 aa, Artificial Sequence
  CDR3
AAEDINYTGTEAYY

SEQ ID NO: 55 - protein, 13 aa, Artificial Sequence
  CDR3
AASNKDYNDYDPD

SEQ ID NO: 56 - protein, 11 aa, Artificial Sequence
  CDR3
AAEDYDTKDRF

SEQ ID NO: 57 - protein, 14 aa, Artificial Sequence
  CDR3
AADKFGADIHEVDY

SEQ ID NO: 58 - protein, 11 aa, Artificial Sequence
  CDR3
AVERYSDQSRF

SEQ ID NO: 59 - protein, 10 aa, Artificial Sequence
  CDR3
AAGDDPKNYD

SEQ ID NO: 60 - protein, 10 aa, Artificial Sequence
  CDR3
HLRVSVTEGY

SEQ ID NO: 61 - protein, 11 aa, Artificial Sequence
  CDR3
AAEDYGLGQRS

SEQ ID NO: 62 - protein, 10 aa, Artificial Sequence
  CDR3
AAGDDPKDYY

SEQ ID NO: 63 - protein, 14 aa, Artificial Sequence
  CDR3
AADRFGAPIHDVDY

SEQ ID NO: 64 - protein, 12 aa, Artificial Sequence
  CDR3
AGETGTYPKPEY

SEQ ID NO: 65 - protein, 19 aa, Artificial Sequence
  CDR3
AADIHCRGYVLFVPSDFGN

SEQ ID NO: 66 - protein, 14 aa, Artificial Sequence
  CDR3
AADKFGADIKEVAY

SEQ ID NO: 67 - protein, 14 aa, Artificial Sequence
  CDR3
AADRFGADIREVDY

SEQ ID NO: 68 - protein, 14 aa, Artificial Sequence
  CDR3
AVEDRQRPGTENYY

SEQ ID NO: 69 - protein, 10 aa, Artificial Sequence
  CDR3
HLRVSVERGY

SEQ ID NO: 70 - protein, 23 aa, Artificial Sequence
  CDR3
QVGQFSSSTTPVQAMSVMSLYAD

SEQ ID NO: 71 - protein, 18 aa, Artificial Sequence
  CDR3
AGTTRSGYVCYDAEPYDS

SEQ ID NO: 72 - protein, 10 aa, Artificial Sequence
  CDR3
AAGDDPKNYS

SEQ ID NO: 73 - protein, 11 aa, Artificial Sequence
  CDR1
GFTLRELDEFA

SEQ ID NO: 74 - protein, 8 aa, Artificial Sequence
  CDR2
ISGTGGIT

SEQ ID NO: 75 - protein, 16 aa, Artificial Sequence
  CDR3
AADERCTDRLIRPPTY

SEQ ID NO: 76 - protein, 121 aa, Artificial Sequence
  MSLN VHH
EVQLVESGGGLVQAGGSLRLSCAASGSIFNINAMGWYRQAPGKEWERELVATISSSNSDNTYYKDSVKGRFTISTNTAKNTWYLQMNSLKPEDTAMYYCAAENYDRKDRYWGQGTQVTVSS

SEQ ID NO: 77 - protein, 121 aa, Artificial Sequence
  MSLN VHH
QVQLVESGGGLVQAGGSLRLSCTASGNIFSINAMGWYRQPPGKEWERELVATISSTNSDNTYYKESVKGRFTISTNTAKNTWYLQMNSLKPEDTAMYYCAAENFDRKDRYWAQGTQVTVSS

SEQ ID NO: 78 - protein, 119 aa, Artificial Sequence
  MSLN VHH
EVQLVESGGGLVQAGGSLRLSCAASESISSIAYMGWYRRISEKERNLVATISSTGSTYYADSVKGRFTISRDNAKNTMYLQMNRLKPEDTAIYYCAASNKAYNDYDPDWGQGTQVTVSS

SEQ ID NO: 79 - protein, 117 aa, Artificial Sequence
  MSLN VHH
EVQLVESGGGWVQSGGSLRLACAASGSSFGLNVVGWYRQAPDKQRELVASIGNGGRTTDYADSVKGRFTISSDNAKNTVFLQMNDLKPEDTAVYYCHLRASVTKGYWGQGTQVTVSS

SEQ ID NO: 80 - protein, 120 aa, Artificial Sequence
  MSLN VHH
QVQLVESGGGLVQAGGSLRLSCAASGSVSSINAMGWYRQGTGEVRKLVATMGSGGNTYYADSVKGRFFITRDYSKNTVSLQMNNLTPEDSATYYCAADRFGASIHEVDYWGKGTLVTVSS

SEQ ID NO: 81 - protein, 127 aa, Artificial Sequence
  MSLN VHH
QVQLVESGGDLVQTGGSLRLSCVVSGSTFAINAMGWYRQAPGKERELVAAISSGGDSTHYADDVKGRFTISRDNAENTMYLQMKSLKPEDTAVYVCNARGCRDFHNPQALCVLRDYWGQGTQVTVSS

SEQ ID NO: 82 - protein, 120 aa, Artificial Sequence
  MSLN VHH
EVQLVESGGGSVQAGGSLKISCAASGSVIDIGAMGWYRHITEKERKLVATINAGGNTYYADSVKGRFTISRDNAKYTVYLQMNSLKPEDTAMYYCAAEDINYTGTEAYYWGQGTQVTVSS

SEQ ID NO: 83 - protein, 119 aa, Artificial Sequence
  MSLN VHH
QVQVVESGGGFVQAGGSLRLSCAASTPIISIAYMGWYRQISEKERQLVATINSGGKTYYADSVKGRFTISRDNAKNTLYLQMNMLKPEDTGMYYCAASNKDYNDYDPDWGQGTQVTVSS

SEQ ID NO: 84 - protein, 121 aa, Artificial Sequence
  MSLN VHH
QVQLVETGGGSVQAGGSLRLSCAASGSIASIDAMGWYRQVPGKEWERELVATISSSNSDNKYYKDSVKGRFTISTNIAKNTWYLQMNNLKPEDTAMYYCAAEDYDTKDRFWGQGTQVTVSS

SEQ ID NO: 85 - protein, 120 aa, Artificial Sequence
  MSLN VHH
EVQLQESGGGLVQAGGSLRLSCAASGAVSSINAMGWYRQTPEKVRKLVATMGSGGNTYYADSVKGRFTISRDYAKNTVALQMNNLIPEDTAVYYCAADKFGADIHEVDYWGKGTLVTVSS

SEQ ID NO: 86 - protein, 119 aa, Artificial Sequence
  MSLN VHH
EVQLVESGGGLVQAGGSLTLSCAASEHTFTIDAMGYYRQIPGRRNERQLVAAAGRTGTTYYNDAVKDRFTIYRDTSKETIILQMNNLRPEDTTMYYCAVERYSDQSRFFGPGTQVTVSS

SEQ ID NO: 87 - protein, 118 aa, Artificial Sequence
  MSLN VHH
EVQLVESGGGLVQPGGSLRLSCVASGSDLSFDAMGWYRQFSATVRERQLVVATSRDGRIYYGDSVKGRFTASRDNLKNSVDLEMNNLKPEDTAIYYCAAGDDPKNYDWGPGTQVTVSS

SEQ ID NO: 88 - protein, 117 aa, Artificial Sequence
  MSLN VHH
EVQLVESGGGWVQSGGSLRLACAASGDSFGLNVVGWYRLAPDKQRELVASIGNGGRTTDYADSVKGRFTISSDNAKNTVFLQMNDLKPEDTAMYYCHLRVSVTEGYWGQGTQVTVSS

SEQ ID NO: 89 - protein, 117 aa, Artificial Sequence
  MSLN VHH
QVQLVESGGGSAQAGGSLILSCVASANLFTIDALGWYRQAPGPKRELVAAISSGGNKYYADAVKGRFTISRDTLTKTMWLQMNNLKPEDTAMYYCAAEDYGLGQRSWGMGTQVTVSS

SEQ ID NO: 90 - protein, 118 aa, Artificial Sequence
  MSLN VHH
QVQLVESGGGLVQAGGSLSLSCVASGDAFSFDAMGWYRQFSGKVNERQLVVATSRDGRTAYGERVKGRFTASRDNSKNTLSLVMNNLQVEDTAIYYCAAGDDPKDYYWGQGTQVTVSS

SEQ ID NO: 91 - protein, 119 aa, Artificial Sequence
  MSLN VHH
QVQLVESGGGLVQAGGSLSLSCAASGSLSSINAMGWYRQLPEMRQLVATMGSDGKTYYADSVKGRFTISRDYAKYTVSLQMNNLRPEDTAIYYCAADRFGAPIHDVDYWGKGTLVTVSV

SEQ ID NO: 92 - protein, 118 aa, Artificial Sequence
  MSLN VHH
EVQLVESGGGLVQAGGSLRLSCSASEKTFSIKYMGYYRQGPGIERKLVATIDTDGKTWYADSVKGRFTISRENGENEIGLEMNRLKPEDTAMYYCAGETGTYPKPEYWGQGTQVTVSS

SEQ ID NO: 93 - protein, 130 aa, Artificial Sequence
  MSLN VHH
QVQLVESGGGLVQAGGSLRLSCAVSGISFEYYAIGWFRQAPGKEREAVSCTTSGTTSGGGVTDYADSLKGRFTISRDVAKNTVYLQMNNLTPEDTAVYYCAADIHCRGYVLFVPSDFGNWGQGTQVTVSS

SEQ ID NO: 94 - protein, 119 aa, Artificial Sequence
  MSLN VHH
EVQLVESGGGTVQPGESLRLSCEASGAVSTINAMGWYRQTPEMRKLVATMGSGGNTYYADSVKGRFTISRDFAGNTVDLQMNDLKPEDTGVYFCAADKFGADIKEVAYWGKGTLVTVSS

SEQ ID NO: 95 - protein, 120 aa, Artificial Sequence
  MSLN VHH
QVQLVESGGGSVQAGGSLTLSCAASGAVSSINAMGWYRQTPEKVRQLVATMGSGGNTYYAASVKGRFTISRDYAKNTVALQMNHLLPEDTAVYYCAADRFGADIREVDYWGKGTQVTVSS

SEQ ID NO: 96 - protein, 124 aa, Artificial Sequence
  MSLN VHH
QVQLVESGGGLVQAGGSLRLSCAASASMGSISNMGWYRQAPGKERGNERNLVATIGSDGRTYYADSVKGRFTISRDNVKNTMILQMNFLKPEDTAMYYCAVEDRQRPGTENYYWGQGTQVTVSS

SEQ ID NO: 97 - protein, 117 aa, Artificial Sequence
  MSLN VHH
EVQLVESGGGLVQAGGSLRLSCAASGSHFGLNVVGWYRQAPGKQRELVASIGNSGRTTDYADSVKGRFTISKDNAQNTIYLQMNNLKPEDTAMYRCHLRVSVERGYWGQGTQVTVSS

SEQ ID NO: 98 - protein, 129 aa, Artificial Sequence
  MSLN VHH
QVQLVESGGGLVQPGGSLRLSCAASGITLDNYAIAWFRQAPGKKREGVSCISSNGNTYYQPSVKGRFTIARDNAKNTVYLHMNNLNPEDTAVYYCQVGQFSSSTTPVQAMSVMSLYADWGQGTQVTVSS

SEQ ID NO: 99 - protein, 125 aa, Artificial Sequence
  MSLN VHH
QVQLVESGGGLVQPGGSLRLSCAASGFTFHYYAIGWFRQAPGKEREGVSCISSSGDSTWFSDSVKGRFTVSRDNAKNIVHLQMNNLKPEDTAVYYCAGTTRSGYVCYDAEPYDSWGQGTQVTVSS

SEQ ID NO: 100 - protein, 118 aa, Artificial Sequence
  MSLN VHH
QVQLVESGGGLVQSGGSLRLSCVASGSAFSFDAMGWYRQFSATRRERQLVVATSRDGRTYYADSVKGRFTATRDNSKNSLYLEMNSLKPEDTAIYYCAAGDDPKNYSWGQGTQVTVSS

SEQ ID NO: 101 - protein, 126 aa, Artificial Sequence
  MSLN VHH
QLQLGASGGGLVQPGGSLRLSCALSGFTLRELDEFAIGWFRQAPGKEREGVSCISGTGGITHYADSVKGRFTISRDIAKTTVYLQMNSLNSEDTAVYYCAADERCTDRLIRPPTYWGQGTQVTVSS

SEQ ID NO: 102 - protein, 126 aa, Artificial Sequence
  MSLN VHH
EVQLVASGGGLVQPGGSLRLSCALSGFTLRELDEFAIGWFRQAPGKEREGVSCISGTGGITHYADSVKGRFTISRDNSKTTVYLQMNSLRAEDTAVYYCAADERCTDRLIRPPTYWGQGTQVTVSS

SEQ ID NO: 103 - protein, 126 aa, Artificial Sequence
  MSLN VHH
QVQLVASGGGLVQPGGSLRLSCALSGFTLRELDEFAIGWFRQAPGKEREGVSCISGTGGITHYADSVKGRFTISRDNSKTTVYLQMNSLRAEDTAVYYCAADERCTDRLIRPPTYWGQGTQVTVSS

SEQ ID NO: 104 - protein, 126 aa, Artificial Sequence
  MSLN VHH
ELQLVASGGGLVQPGGSLRLSCALSGFTLRELDEFAIGWFRQAPGKEREGVSCISGTGGITHYADSVKGRFTISRDNSKTTVYLQMNSLRAEDTAVYYCAADERCTDRLIRPPTYWGQGTQVTVSS

SEQ ID NO: 105 - protein, 126 aa, Artificial Sequence
  MSLN VHH
EVQLGASGGGLVQPGGSLRLSCALSGFTLRELDEFAIGWFRQAPGKEREGVSCISGTGGITHYADSVKGRFTISRDNSKTTVYLQMNSLRAEDTAVYYCAADERCTDRLIRPPTYWGQGTQVTVSS

SEQ ID NO: 106 - protein, 126 aa, Artificial Sequence
  MSLN VHH
EVQLVASGGGLVQPGGSLRLSCALSGFTLRELDEFAIGWFRQAPGKEREGVSCISGTGGITHYADSVKGRFTISRDNSKTTVYLQMNSLNAEDTAVYYCAADERCTDRLIRPPTYWGQGTQVTVSS

SEQ ID NO: 107 - protein, 126 aa, Artificial Sequence
  MSLN VHH
EVQLVASGGGLVQPGGSLRLSCALSGFTLRELDEFAIGWFRQAPGKEREGVSCISGTGGITHYADSVKGRFTISRDNSKTTVYLQMNSLRSEDTAVYYCAADERCTDRLIRPPTYWGQGTQVTVSS

SEQ ID NO: 108 - protein, 126 aa, Artificial Sequence
  MSLN VHH
ELQLGASGGGLVQPGGSLRLSCALSGFTLRELDEFAIGWFRQAPGKEREGVSCISGTGGITHYADSVKGRFTISRDNSKTTVYLQMNSLRAEDTAVYYCAADERCTDRLIRPPTYWGQGTQVTVSS

SEQ ID NO: 109 - protein, 126 aa, Artificial Sequence
  MSLN VHH
QLQLGESGGGLVQPGGSLRLSCALSGFTLRELDEFAIGWFRQAPGKEREGVSCISGTGGITHYADSVKGRFTISRDIAKTTVYLQMNSLNSEDTAVYYCAADERCTDRLIRPPTYWGQGTQVTVSS

SEQ ID NO: 110 - protein, 126 aa, Artificial Sequence
  MSLN VHH
QLQLVASGGGLVQPGGSLRLSCALSGFTLRELDEFAIGWFRQAPGKEREGVSCISGTGGITHYADSVKGRFTISRDIAKTTVYLQMNSLNSEDTAVYYCAADERCTDRLIRPPTYWGQGTQVTVSS

SEQ ID NO: 111 - protein, 126 aa, Artificial Sequence
  MSLN VHH
QLQLVESGGGLVQPGGSLRLSCALSGFTLRELDEFAIGWFRQAPGKEREGVSCISGTGGITHYADSVKGRFTISRDIAKTTVYLQMNSLNSEDTAVYYCAADERCTDRLIRPPTYWGQGTQVTVSS

SEQ ID NO: 112 - protein, 126 aa, Artificial Sequence
  MSLN VHH
QLQLGASGGGLVQPGGSLRLSCAASGFTLRELDEFAIGWFRQAPGKEREGVSCISGTGGITHYADSVKGRFTISRDIAKTTVYLQMNSLNSEDTAVYYCAADERCTDRLIRPPTYWGQGTQVTVSS

SEQ ID NO: 113 - protein, 126 aa, Artificial Sequence
  MSLN VHH
EVQLGASGGGLVQPGGSLRLSCALSGFTLRELDEFAIGWFRQAPGKEREGVSCISGTGGITHYADSVKGRFTISRDIAKTTVYLQMNSLNSEDTAVYYCAADERCTDRLIRPPTYWGQGTQVTVSS

SEQ ID NO: 114 - protein, 126 aa, Artificial Sequence
  MSLN VHH
QLQLGASGGGLVQPGGSLRLSCALSGFTLRELDEFAIGWFRQAPGKEREGVSCISGTGGITHYADSVKGRFTISRDNSKTTVYLQMNSLNSEDTAVYYCAADERCTDRLIRPPTYWGQGTQVTVSS

SEQ ID NO: 115 - protein, 126 aa, Artificial Sequence
  MSLN VHH
QLQLGASGGGLVQPGGSLRLSCALSGFTLRELDEFAIGWFRQAPGKEREGVSCISGTGGITHYADSVKGRFTISRDIAKNTVYLQMNSLNSEDTAVYYCAADERCTDRLIRPPTYWGQGTQVTVSS

SEQ ID NO: 116 - protein, 126 aa, Artificial Sequence
  MSLN VHH
QLQLGASGGGLVQPGGSLRLSCALSGFTLRELDEFAIGWFRQAPGKEREGVSCISGTGGITHYADSVKGRFTISRDIAKTTLYLQMNSLNSEDTAVYYCAADERCTDRLIRPPTYWGQGTQVTVSS

SEQ ID NO: 117 - protein, 126 aa, Artificial Sequence
  MSLN VHH
QLQLGASGGGLVQPGGSLRLSCALSGFTLRELDEFAIGWFRQAPGKEREGVSCISGTGGITHYADSVKGRFTISRDIAKTTVYLQMNSLRAEDTAVYYCAADERCTDRLIRPPTYWGQGTQVTVSS

SEQ ID NO: 118 - protein, 126 aa, Artificial Sequence
  MSLN VHH
ELQLGASGGGLVQPGGSLRLSCALSGFTLRELDEFAIGWFRQAPGKEREGVSCISGTGGITHYADSVKGRFTISRDNSKNTLYLQMNSLRAEDTAVYYCAADERCTDRLIRPPTYWGQGTQVTVSS

SEQ ID NO: 119 - protein, 126 aa, Artificial Sequence; identical to SEQ ID NO: 115
  MSLN VHH

SEQ ID NO: 120 - protein, 126 aa, Artificial Sequence; identical to SEQ ID NO: 116
  MSLN VHH

SEQ ID NO: 121 - protein, 229 aa, Artificial Sequence
  CH
ESKYGPPCPPCPAPEFLGGPSVFLFPPKPKDTLMISRTPEVTCVVVDVSQEDPEVQFNWYVDGVEVHNAKTKPREEQFNSTYRVVSVLTVLHQDWLNGKEYKCKVSNKGLPSSIEKTISKAKGQPREPQVYTLPPSQEEMTKNQVSLTCLVKGFYPSDIAVEWESNGQPENNYKTTPPVLDSDGSFFLYSRLTVDKSRWQEGNVFSCSVMHEALHNHYTQKSLSLSLGK

SEQ ID NO: 122 - DNA, 24 bp, Artificial Sequence
  primer
gtcctggctgctcttctacaaggc

SEQ ID NO: 123 - DNA, 23 bp, Artificial Sequence
  primer
ggtacgtgctgttgaactgttcc

SEQ ID NO: 124 - DNA, 29 bp, Artificial Sequence
  primer
gatgtgcagctgcaggagtctggrggagg

SEQ ID NO: 125 - DNA, 35 bp, Artificial Sequence
  primer
ggactagtgcggccgctggagacggtgacctgggt